European Patent Application EP 4 417 686 A2, published August 21, 2024. Title: POLYPEPTIDES, NUCLEIC ACID MOLECULES, CELLS, AND RELATED METHODS. Applicant: CHILDREN'S HOSPITAL MEDICAL CENTER. The sequence listing filed with the application follows.

SEQUENCE LISTING (65 sequences)

SEQ ID NO: 1 - DNA, 20 bp, synthetic construct
  misc_feature 1..20: note = Primer a - exon 3 Gm7325
  source 1..20: mol_type = other DNA
gcagcgatcgaagcaccatc

SEQ ID NO: 2 - DNA, 20 bp, synthetic construct
  misc_feature 1..20: note = Primer b - exon 3 of Gm7325
  source 1..20: mol_type = other DNA
gaggcctctccagaatccgg

SEQ ID NO: 3 - DNA, 20 bp, synthetic construct
  misc_feature 1..20: note = Primer 1a - Table E1
  source 1..20: mol_type = other DNA
gaagggaggactccacaccc

SEQ ID NO: 4 - DNA, 20 bp, synthetic construct
  misc_feature 1..20: note = Primer 1b - Table E1
  source 1..20: mol_type = other DNA
cgcctggactaaccggctcc

SEQ ID NO: 5 - DNA, 21 bp, synthetic construct
  misc_feature 1..21: note = Primer 2a - Table E1
  source 1..21: mol_type = other DNA
agtgatgctgaatccaccgca

SEQ ID NO: 6 - DNA, 21 bp, synthetic construct
  misc_feature 1..21: note = Primer 2b - Table E1
  source 1..21: mol_type = other DNA
ccaataacaacacactgtcct

SEQ ID NO: 7 - DNA, 22 bp, synthetic construct
  misc_feature 1..22: note = Primer 3a - Table E1
  source 1..22: mol_type = other DNA
atgccagaagaaagctgcactg

SEQ ID NO: 8 - DNA, 22 bp, synthetic construct
  misc_feature 1..22: note = Primer 3b - Table E1
  source 1..22: mol_type = other DNA
tcacttctgggggcccaatctc

SEQ ID NO: 9 - DNA, 22 bp, synthetic construct
  misc_feature 1..22: note = Primer 4a - Table E1
  source 1..22: mol_type = other DNA
atgcccgttccattgctcccga

SEQ ID NO: 10 - DNA, 22 bp, synthetic construct
  misc_feature 1..22: note = Primer 4b - Table E1
  source 1..22: mol_type = other DNA
tcacttctgggggcccaatctc

SEQ ID NO: 11 - DNA, 20 bp, synthetic construct
  misc_feature 1..20: note = Primer 5a - Table E1
  source 1..20: mol_type = other DNA
caggagggcaagaagttcag

SEQ ID NO: 12 - DNA, 20 bp, synthetic construct
  misc_feature 1..20: note = Primer 5b - Table E1
  source 1..20: mol_type = other DNA
atgtcttgggagctcagtcg

SEQ ID NO: 13 - DNA, 20 bp, synthetic construct
  misc_feature 1..20: note = Primer 6a - Table E1
  source 1..20: mol_type = other DNA
accagctttcatgccagaag

SEQ ID NO: 14 - DNA, 20 bp, synthetic construct
  misc_feature 1..20: note = Primer 6b - Table E1
  source 1..20: mol_type = other DNA
atgtcttgggagctcagtcg

SEQ ID NO: 15 - DNA, 19 bp, synthetic construct
  misc_feature 1..19: note = Primer 7a - Table E1
  source 1..19: mol_type = other DNA
atcgctaccaagaggcgtt

SEQ ID NO: 16 - DNA, 20 bp, synthetic construct
  misc_feature 1..20: note = Primer 7b - Table E1
  source 1..20: mol_type = other DNA
cacagcacagacaaaccagg

SEQ ID NO: 17 - DNA, 20 bp, synthetic construct
  misc_feature 1..20: note = Primer 8a - Table E1
  source 1..20: mol_type = other DNA
ttagtggtccctggatgctc

SEQ ID NO: 18 - DNA, 20 bp, synthetic construct
  misc_feature 1..20: note = Primer 8b - Table E1
  source 1..20: mol_type = other DNA
gacgcaccaatgtgagaaaa

SEQ ID NO: 19 - DNA, 19 bp, synthetic construct
  misc_feature 1..19: note = Primer 9a - Table E1
  source 1..19: mol_type = other DNA
ggggacgagttctccttcg

SEQ ID NO: 20 - DNA, 21 bp, synthetic construct
  misc_feature 1..21: note = Primer 9b - Table E1
  source 1..21: mol_type = other DNA
tgcttctgcgtgcttcattag

SEQ ID NO: 21 - DNA, 20 bp, synthetic construct
  misc_feature 1..20: note = Primer 10a - Table E1
  source 1..20: mol_type = other DNA
ggctctcttcggagctttgg

SEQ ID NO: 22 - DNA, 21 bp, synthetic construct
  misc_feature 1..21: note = Primer 10b - Table E1
  source 1..21: mol_type = other DNA
ggtggctgattggtgtaccag

SEQ ID NO: 23 - DNA, 20 bp, synthetic construct
  misc_feature 1..20: note = Primer 11a - Table E1
  source 1..20: mol_type = other DNA
ctacaggccttgctcagctc

SEQ ID NO: 24 - DNA, 20 bp, synthetic construct
  misc_feature 1..20: note = Primer 11b - Table E1
  source 1..20: mol_type = other DNA
gtgggagttgcattcactgg

SEQ ID NO: 25 - DNA, 20 bp, synthetic construct
  misc_feature 1..20: note = Primer 12a - -Table E1
  source 1..20: mol_type = other DNA
acctccacagcacagacaga

SEQ ID NO: 26 - DNA, 20 bp, synthetic construct
  misc_feature 1..20: note = Primer 12b - Table E1
  source 1..20: mol_type = other DNA
cagcttgaacttgttgtggg

SEQ ID NO: 27 - DNA, 20 bp, synthetic construct
  misc_feature 1..20: note = Primer 13a - Table E1
  source 1..20: mol_type = other DNA
gcaggacttggtggacaaac

SEQ ID NO: 28 - DNA, 20 bp, synthetic construct
  misc_feature 1..20: note = Primer 13b - Table E1
  source 1..20: mol_type = other DNA
acttggccaggttgacattg

SEQ ID NO: 29 - DNA, 20 bp, synthetic construct
  misc_feature 1..20: note = Primer 14a - Table E1
  source 1..20: mol_type = other DNA
tgcgacttcaacagcaactc

SEQ ID NO: 30 - DNA, 20 bp, synthetic construct
  misc_feature 1..20: note = Primer 14b - Table E1
  source 1..20: mol_type = other DNA
gcctctcttgctcagtgtcc

SEQ ID NO: 31 - protein, 16 aa, synthetic construct
  REGION 1..16: note = Mouse myomaker polypeptide with modifications (e.g., deletions)
MKEKKGLYPDKSIYTQ

SEQ ID NO: 32 - protein, 108 aa, synthetic construct
  REGION 1..108: note = Myomerger mouse-long
MPEESCTVKLIQLKTGEYRGAGPAMPVPLLPMVLRSLLSRLLLPVARLARQHLLPLLRRLARRLSSQDMREALLSCLLFVLSQQQPPDSGEASRVDHSQRKERLGPQK

SEQ ID NO: 33 - protein, 84 aa, synthetic construct
  REGION 1..84: note = Myomerger - Mouse (short)
MPVPLLPMVLRSLLSRLLLPVARLARQHLLPLLRRLARRLSSQDMREALLSCLLFVLSQQQPPDSGEASRVDHSQRKERLGPQK

SEQ ID NO: 34 - protein, 84 aa, synthetic construct
  REGION 1..84: note = Myomerger - Human
MPTPLLPLLLRLLLSCLLLPAARLARQYLLPLLRRLARRLGSQDMREALLGCLLFILSQRHSPDAGEASRVDRLERRERLGPQK

SEQ ID NO: 35 - protein, 84 aa, synthetic construct
  REGION 1..84: note = Myomerger - Cat
MPAPLLPLLLRTLMSRLLLPATRLARRHLLPLLRRLARRLGSQDVREALLGCLLFILSQSRPPDAEEVSRVAGQERRERLAPPK

SEQ ID NO: 36 - protein, 85 aa, synthetic construct
  REGION 1..85: note = Myomerger - Rabbit
MPAPLLPLLLRTLLSRLLLPAARLARRHLLPLLRRLAQRLGSQGTREALLGCLLFVLSQRQPPDASGEASRVDPPERKERLGRQK

SEQ ID NO: 37 - protein, 84 aa, synthetic construct
  REGION 1..84: note = Myomerger - Dog
MPAPLLPLLLRTLVSRLLLPAARLARRHLLPLLRGLARRLGSQEVREALLGCLLFILSQRHPPDAEEASRVAGQERKERLAPPK

SEQ ID NO: 38 - protein, 84 aa, synthetic construct
  REGION 1..84: note = Myomerger - Elephant
MPVPLLSLLLRALLSRLLLPAARLARQHLLPLLRRLARRLGSQDMRQALLGCLLFVLSQQHPPDAGEASREALSERRGRLAPQK

SEQ ID NO: 39 - DNA, 327 bp, synthetic construct
  misc_feature 1..327: note = Myomerger - Mouse (long) cDNA
  source 1..327: mol_type = other DNA
atgccagaagaaagctgcactgtaaaactaatccagttgaaaactggggagtacagaggtgcaggtcctgccatgcccgttccattgctcccgatggtgcttcgatcgctgctgtcccgcctgctgctgcctgttgcccgcctggcccggcagcacctcctgcccttgctgcgccggctggcccgccgactgagctcccaagacatgagagaggctctgctgagctgtctgctctttgtcctcagccagcaacagccaccggattctggagaggcctccagagtggaccactcccagaggaaggagagattgggcccccagaagtga

SEQ ID NO: 40 - DNA, 255 bp, synthetic construct
  misc_feature 1..255: note = Myomerger - Mouse (short) cDNA
  source 1..255: mol_type = other DNA
atgcccgttccattgctcccgatggtgcttcgatcgctgctgtcccgcctgctgctgcctgttgcccgcctggcccggcagcacctcctgcccttgctgcgccggctggcccgccgactgagctcccaagacatgagagaggctctgctgagctgtctgctctttgtcctcagccagcaacagccaccggattctggagaggcctccagagtggaccactcccagaggaaggagagattgggcccccagaagtga

SEQ ID NO: 41 - DNA, 255 bp, synthetic construct
  misc_feature 1..255: note = Myomerger - Human cDNA
  source 1..255: mol_type = other DNA
atgcccacgccactgctcccgctgctgcttcgattgctgctgtcctgcctgctgctgcctgctgcccgcctggcccgccaatacctcctgcccctgctgcgccgattggcccgccgcctgggctcccaggacatgcgagaggctttgctgggctgtctgctgttcattctcagccagcgacactcgccagacgctggggaggcctcaagagtggaccgcctggagaggagggagaggttaggcccccaaaagtga

SEQ ID NO: 42 - DNA, 255 bp, synthetic construct
  misc_feature 1..255: note = Myomerger - Cat cDNA
  source 1..255: mol_type = other DNA
atgcccgctccactgctcccactgctgcttcgaaccctgatgtcccgcttgctgctgcctgccacccgcctggcccgccggcacctcctgcccctcctgcgccgactggcccgccgcctgggctcgcaggatgttcgagaagctttgctgggctgtctgttgttcatcctcagccagagccgcccgcccgacgctgaggaggtctccagagtggctggccaggagaggagggagaggctagctcccccaaaatga

SEQ ID NO: 43 - DNA, 258 bp, synthetic construct
  misc_feature 1..258: note = Myomerger - Rabbit cDNA
  source 1..258: mol_type = other DNA
atgcctgcccccctgctgccgctgctgctgcgaacgctgctgtcccgtctgctgctgcccgctgcccgcctggcccgccggcacctcctgcccctgctgcgccgactggctcaacgcctgggctcccagggcacgcgcgaggctttgctgggctgtttgctgtttgtcctcagccagagacagccgccagatgcctctggggaggcctccagagtggacccaccggagaggaaggagaggttaggccgccaaaagtga

SEQ ID NO: 44 - DNA, 255 bp, synthetic construct
  misc_feature 1..255: note = Myomerger - Dog cDNA
  source 1..255: mol_type = other DNA
atgcctgctccactgctcccactgctgctgcgaacgctggtgtctcgcctgctgctgcctgctgcccgcctggcccggcggcacctcctgcccctgctgcgtggactggcccgccgcctaggctcgcaggaggttcgagaggctttgctgggctgtctgttgttcatcctcagccagagacatccgccggacgccgaggaggcctccagagtggctggccaggagaggaaggagaggctagctccccccaaatga

SEQ ID NO: 45 - DNA, 255 bp, synthetic construct
  misc_feature 1..255: note = Myomerger - Elephant cDNA
  source 1..255: mol_type = other DNA
atgcccgtcccgctgctctcgctgctgctgcgcgcgctgctgtcccgcctgctgctgcctgctgcccgcctggcccgccagcacctcctgcccctcctgcgccgacttgctcgccgcctgggctcccaggacatgcgacaggctctcttgggatgtctgctctttgtcctcagccagcaacacccgccggacgctggtgaggcctccagagaggccctctcagagaggagagggaggctagccccccaaaagtga

SEQ ID NO: 46 - DNA, 1275 bp, synthetic construct
  misc_feature 1..1275: note = Myomerger - Human (+strand)
  source 1..1275: mol_type = other DNA
ctgcccggtgagagctgccgtggattggtgggggtaggggactgagaggtcagggagtgtcaggtcagggtggatcaggagccccaaaagaaaaattgagaattgcctggagaagaactcctgctagactgagggagaagggttagggaactccaggggcattgaggctgtgcaagaggagggggtgactagaggaagggaggggccagggagcagtaggaatgcctggagctgggaacggcaagctgtaggtcttggtttactcttgccttggttcagtctccccatctgtgctatggtgagaaccttcctgcctcagctgccttgccaagagaaagggcttcatgaaagcaaaaatgacctacaaattgaggtcaggagcaggaaggtgtaaactgaagggagggggaactcctgcccaccccatgtccttgccaggtgaggcagaaccaggacatgcaagcctaaagtctgtgttgtcttcccaggcactgactcactggccctgccatgcccacgccactgctcccgctgctgcttcgattgctgctgtcctgcctgctgctgcctgctgcccgcctggcccgccaatacctcctgcccctgctgcgccgattggcccgccgcctgggctcccaggacatgcgagaggctttgctgggctgtctgctgttcattctcagccagcgacactcgccagacgctggggaggcctcaagagtggaccgcctggagaggagggagaggttaggcccccaaaagtgaggccacaagtcctggcagcagctgtatccacaaaatgctttcttttggagtaggataatcctggcaccagcactgaccgaagcctgcccagtggacagaagatatagtgagggttgtgcatgagagggatctgccacagacatgcctctccactcccaacagaaatgtctttctggaagaatgccttgcatctagcacaaaactgattattgcccctctgtcctccagcagttcctcccaaagaccactcctaatcacctctggcctcaggcgggaggggaactaacacccacccacccctgccctccctgcaaatgggaacatcaaggttcccagtgcttaactgagggacaagtgacaatttagcagagaggcaagatttgaatccagactgtcttccagactcaggacctaccttaaaataatatctgagttgcttatggaggcagacctgcctgcaaagcccagcactcagcaagtgctcaataaatatttgatttgaattctttc

SEQ ID NO: 47 - DNA, 1275 bp, synthetic construct
  misc_feature 1..1275: note = Myomerger - Human (- strand, reverse complement)
  source 1..1275: mol_type = other DNA
gaaagaattcaaatcaaatatttattgagcacttgctgagtgctgggctttgcaggcaggtctgcctccataagcaactcagatattattttaaggtaggtcctgagtctggaagacagtctggattcaaatcttgcctctctgctaaattgtcacttgtccctcagttaagcactgggaaccttgatgttcccatttgcagggagggcaggggtgggtgggtgttagttcccctcccgcctgaggccagaggtgattaggagtggtctttgggaggaactgctggaggacagaggggcaataatcagttttgtgctagatgcaaggcattcttccagaaagacatttctgttgggagtggagaggcatgtctgtggcagatccctctcatgcacaaccctcactatatcttctgtccactgggcaggcttcggtcagtgctggtgccaggattatcctactccaaaagaaagcattttgtggatacagctgctgccaggacttgtggcctcacttttgggggcctaacctctccctcctctccaggcggtccactcttgaggcctccccagcgtctggcgagtgtcgctggctgagaatgaacagcagacagcccagcaaagcctctcgcatgtcctgggagcccaggcggcgggccaatcggcgcagcaggggcaggaggtattggcgggccaggcgggcagcaggcagcagcaggcaggacagcagcaatcgaagcagcagcgggagcagtggcgtgggcatggcagggccagtgagtcagtgcctgggaagacaacacagactttaggcttgcatgtcctggttctgcctcacctggcaaggacatggggtgggcaggagttccccctcccttcagtttacaccttcctgctcctgacctcaatttgtaggtcatttttgctttcatgaagccctttctcttggcaaggcagctgaggcaggaaggttctcaccatagcacagatggggagactgaaccaaggcaagagtaaaccaagacctacagcttgccgttcccagctccaggcattcctactgctccctggcccctcccttcctctagtcaccccctcctcttgcacagcctcaatgcccctggagttccctaacccttctccctcagtctagcaggagttcttctccaggcaattctcaatttttcttttggggctcctgatccaccctgacctgacactccctgacctctcagtcccctacccccaccaatccacggcagctctcaccgggcag

SEQ ID NO: 48 - DNA, 1136 bp, synthetic construct
  misc_feature 1..1136: note = Myomerger - Mouse (+strand)
  source 1..1136: mol_type = other DNA
ccaataacaacacactgtcctcgtttattgactacctgctgcgtaccaagctttgaaagtactcattctttaacgggaagcaagggcttataattttaaggtagacgggacagtttggatttaaataccacctcttagctaaattgtcttgagtctaagtgaaacatcatctcttaactgaccttgatacccgcatttgcaggtccaccctggaggccagagataaggcagagggagctgcagagaggaagggtcaatcaacacaatctgtagcctgctaggagctaggggagtgggaactgttcaggtcagagccctcttgcactcagcccggactgtcttcgcccactgggcagtctgccgtccatgcccgtgcgtgcggaccgacgcctggactaaccggctccaaaagtactttgatgggcgttgctgtttccaggacccgtggcctcacttctgggggcccaatctctccttcctctgggagtggtccactctggaggcctctccagaatccggtggctgttgctggctgaggacaaagagcagacagctcagcagagcctctctcatgtcttgggagctcagtcggcgggccagccggcgcagcaagggcaggaggtgctgccgggccaggcgggcaacaggcagcagcaggcgggacagcagcgatcgaagcaccatcgggagcaatggaacgggcatggcaggacctgcacctgcaaagggaacccgggttttagactgtacctcaggcacgcacctcacctggcaaagcagggtgcgggggtgtggagtcctcccttcagcttatacctctgtactccccagttttcaactggattagttttacagtgcagctttcttctggcatgaaagctggttaaggagttcactcactgttatcacagatgggaagggagcccagggctggaaggtggtggggactgaggctagggccttttccagaacccacttcctttaatccctccctccctttgcatactctgacctgaagcctgaacttcttgccctcctgctcaccagttctaaccggccagtggcagctctcaccagtcagaactgctcagaatcaatttcaggatgcttttgcctgcggtggattcagcatcact

SEQ ID NO: 49 - DNA, 1136 bp, synthetic construct
  misc_feature 1..1136: note = Myomerger - Mouse (- strand, reverse complement)
  source 1..1136: mol_type = other DNA
agtgatgctgaatccaccgcaggcaaaagcatcctgaaattgattctgagcagttctgactggtgagagctgccactggccggttagaactggtgagcaggagggcaagaagttcaggcttcaggtcagagtatgcaaagggagggagggattaaaggaagtgggttctggaaaaggccctagcctcagtccccaccaccttccagccctgggctcccttcccatctgtgataacagtgagtgaactccttaaccagctttcatgccagaagaaagctgcactgtaaaactaatccagttgaaaactggggagtacagaggtataagctgaagggaggactccacacccccgcaccctgctttgccaggtgaggtgcgtgcctgaggtacagtctaaaacccgggttccctttgcaggtgcaggtcctgccatgcccgttccattgctcccgatggtgcttcgatcgctgctgtcccgcctgctgctgcctgttgcccgcctggcccggcagcacctcctgcccttgctgcgccggctggcccgccgactgagctcccaagacatgagagaggctctgctgagctgtctgctctttgtcctcagccagcaacagccaccggattctggagaggcctccagagtggaccactcccagaggaaggagagattgggcccccagaagtgaggccacgggtcctggaaacagcaacgcccatcaaagtacttttggagccggttagtccaggcgtcggtccgcacgcacgggcatggacggcagactgcccagtgggcgaagacagtccgggctgagtgcaagagggctctgacctgaacagttcccactcccctagctcctagcaggctacagattgtgttgattgacccttcctctctgcagctccctctgccttatctctggcctccagggtggacctgcaaatgcgggtatcaaggtcagttaagagatgatgtttcacttagactcaagacaatttagctaagaggtggtatttaaatccaaactgtcccgtctaccttaaaattataagcccttgcttcccgttaaagaatgagtactttcaaagcttggtacgcagcaggtagtcaataaacgaggacagtgtgttgttattgg

SEQ ID NO: 50 - protein, 221 aa, synthetic construct
  REGION 1..221: note = Myomaker - Human
MGTLVAKLLLPTLSSLAFLPTVSIAAKRRFHMEAMVYLFTLFFVALHHACNGPGLSVLCFMRHDILEYFSVYGTALSMWVSLMALADFDEPKRSTFVMFGVLTIAVRIYHDRWGYGVYSGPIGTAILIIAAKWLQKMKEKKGLYPDKSVYTQQIGPGLCFGALALMLRFFFEDWDYTYVHSFYHCALAMSFVLLLPKVNKKAGSPGTPAKLDCSTLCCACV

SEQ ID NO: 51 - protein, 221 aa, synthetic construct
  REGION 1..221: note = Myomaker - Dog
MGTLAAKLLLPTLSSLAFLPTVSIAAKRRFHMEAMVYLFTMFFVALHHACNGPGLSVLCFMRHDVLEYFSVYGTALSMWVSLMALADFDEPKRSTFVMFGVLTIAVRIYHDRWGYGVYSGPIGTAVLIIATKWLQQMKEKKSLYPDKSVYTQQIGPGLCFGALALMLRFFFEDWDYTYVHSFYHCALAMSFVLLLPKVNKKAGSAGPPAKLDCSTLCCACI

SEQ ID NO: 52 - protein, 221 aa, synthetic construct
  REGION 1..221: note = Myomaker - Pig
MGTVMAKLLLPTLSSLAFLPTVSIAAKRRFHMEAMVYLFTTFFVAFYHACHGPGLAMICFLRLDILEYFSVYGTALSMWVSLMALADFDEPKRSTFVMFGVLTIAVRIYHDRWGYGVYSGPIGTAALIIAAKWLQQMKDQRRLYPDKSVYTQQIGPGLCFGALALMLRFFFEEWDYTYVHSFYHCALAMSFVLLLPKANKKAGSAGPPAKLDCSTLCCACI

SEQ ID NO: 53 - protein, 221 aa, synthetic construct
  REGION 1..221: note = Myomaker - Mouse
MGTVVAKLLLPTLSSLAFLPTVSIATKRRFYMEAMVYLFTMFFVAFSHACDGPGLSVLCFMRRDILEYFSIYGTALSMWVSLMALADFDEPQRSTFTMLGVLTIAVRTFHDRWGYGVYSGPIGTATLIIAVKWLKKMKEKKGLYPDKSIYTQQIGPGLCFGALALMLRFFFEEWDYTYVHSFYHCALAMSFVLLLPKVNKKAGNAGAPAKLTFSTLCCTCV

SEQ ID NO: 54 - protein, 221 aa, synthetic construct
  REGION 1..221: note = Myomaker - Opossum
MGTLVTKLLLPTISSLAFLPTISIAAKRRFHMEAMVYLFTMFFIAIYHACDGPGLSVLCFMRYDILEYFSIYGTALSMWVSLMALAEFDEPKRSTFVMFGVLTIAVRIYQDRWGYGVYSGPIGTAVLIIATKWLQKMKEKKGLYPDKSVYTQQIGPGFCFGALALMLRFFFQEWDYTYVHSFYHCSLAMSFVLLLPKVNKKAGNAGTPAKLDCSTLCCACI

SEQ ID NO: 55 - protein, 220 aa, synthetic construct
  REGION 1..220: note = Myomaker - Zebrafish
MGAFIAKMLLPTISSLVFVPAASVAAKRGFHMEAMVYFFTMFFTAIYHACDGPGLSILCFMKYDILEYFSVYGTAISMWVTLLALGDFDEPKRSSLTMFGVLTAAVRIYQDRLGYGIYSGPIGTAVFMITVKWLQKMKEKKGLYPDKSVYTQQVGPGCCFGALALMLRFYFEEWDYAYVHSFYHVSLAMSFILLLPKKNRYAGTGRNAAKLNCYTLCCCV

SEQ ID NO: 56 - DNA, 666 bp, synthetic construct
  misc_feature 1..666: note = Myomaker - Human cDNA
  source 1..666: mol_type = other DNA
atggggacgctggtggccaagctgctcctgcccaccctcagcagcctggccttcctccccactgtcagcatcgcggccaagaggcggttccacatggaggccatggtctacctcttcaccctgttcttcgtggcgctccaccatgcctgcaatggacccggcttgtctgtgctgtgcttcatgcgtcacgacatcctggagtatttcagtgtctacgggacagccctgagcatgtgggtctcgctgatggcactggccgacttcgacgaacccaagaggtcaacatttgtgatgttcggcgtcctgaccattgctgtgcggatctaccatgaccgatggggctacggggtgtactcgggccccatcggcacagccatcctcatcatcgcggcaaagtggctacagaagatgaaggagaagaagggcctgtacccagacaagagcgtctacacccagcagataggccccggcctctgcttcggggcgctggccctgatgctacgcttcttctttgaggactgggactacacttatgtccacagcttctaccactgtgccctggctatgtcctttgttctgctgctgcccaaggtcaacaagaaggctggatccccggggaccccggccaagctggactgctccaccctgtgctgtgcttgtgtctga

SEQ ID NO: 57 - DNA, 666 bp, synthetic construct
  misc_feature 1..666: note = Myomaker - Dog cDNA
  source 1..666: mol_type = other DNA
atggggacgctcgcggcgaagctgctcctgcccaccctcagcagcctggccttcctccccaccgtcagcatcgccgccaagcggcggttccacatggaggccatggtctacctcttcaccatgttcttcgtggcactccaccacgcgtgcaacgggcccgggctatcggtgctctgcttcatgcgccacgacgtcctggagtacttcagcgtctatgggacggcactgagcatgtgggtctcgctgatggcactggctgacttcgacgaacccaagaggtcgacttttgtgatgtttggcgtcctgaccatcgccgtgcggatctaccatgaccgctggggctacggggtgtactcgggccccattggcacggctgtcctcatcatcgccacaaagtggctgcagcagatgaaggagaagaagagtctgtacccggacaagagtgtctacacccagcagataggccctggcctctgttttggggcactggcccttatgctgcgcttcttttttgaggactgggattacacctatgtccacagcttctaccactgtgccctggccatgtccttcgtcctcctgctccccaaggtcaacaagaaggctggaagcgcggggccccctgccaagctagactgctctaccctttgctgtgcttgcatctga

SEQ ID NO: 58 - DNA, 666 bp, synthetic construct
  misc_feature 1..666: note = Myomaker - Pig cDNA
  source 1..666: mol_type = other DNA
atggggaccgtcatggccaaactgctgctacccacgctgagcagcctggccttcctccccacggtcagcatcgctgccaagcggcggttccacatggaggccatggtctatctcttcaccacgttcttcgtggcgttctaccacgcctgccacgggccgggcctggctatgatctgctttctgcgccttgacatcctggagtatttcagcgtctacggaaccgccctgagcatgtgggtctcgctgatggcgctggctgacttcgacgagcccaagaggtcgactttcgtgatgtttggcgtcctgaccatcgccgtgcggatctaccacgaccgctggggctacggcgtgtactcgggccccatcggcacggccgccctcatcatcgcggccaagtggctgcagcagatgaaggaccaacggcgcctgtatccagacaagagcgtgtacacacagcagataggccccggcctctgcttcggggcgctggccctcatgctgcgctttttcttcgaggagtgggattatacctacgtccacagcttctaccactgcgccctggccatgtccttcgtcctgctgctgcccaaggccaacaagaaggctggaagcgcagggccacccgccaagctggactgctccaccctctgctgtgcttgtatctga

SEQ ID NO: 59 - DNA, 666 bp, synthetic construct
  misc_feature 1..666: note = Myomaker - Mouse cDNA
  source 1..666: mol_type = other DNA
atggggacagttgtagccaaactgctcctgcctaccctcagcagcctggccttcctcccgacagtgagcatcgctaccaagaggcgtttctacatggaggccatggtctacctcttcaccatgttctttgtggcgttctcccatgcctgtgatgggcctggtttgtctgtgctgtgcttcatgcgccgtgacattctggagtacttcagcatctatggaacagccctgagcatgtgggtctccctgatggcactggccgactttgatgaaccccagagatcgaccttcacaatgcttggcgtccttaccatcgctgtgcggacttttcatgaccgctggggttacggggtatactccggtcccataggcacggccaccctcatcattgctgtaaagtggctgaagaagatgaaagagaagaagggcctgtaccccgacaagagcatctacacccagcagataggccccggcctgtgctttggggccctggccctgatgcttcgattcttctttgaggaatgggattacacctacgtccacagcttctaccactgtgccctggccatgtcctttgtcctgctgctgcccaaggtcaacaagaaggctgggaacgcaggggcccccgccaagctgaccttctccaccctctgctgcacttgtgtctga

SEQ ID NO: 60 - DNA, 666 bp, synthetic construct
  misc_feature 1..666: note = Myomaker - Opossum cDNA
  source 1..666: mol_type = other DNA
atggggactcttgttaccaagttgcttcttcccacaatcagcagcctcgcctttctccccaccatcagcatcgctgctaagaggagattccacatggaagccatggtctacctcttcaccatgttcttcatagcaatatatcatgcatgtgacgggccaggcttatcagtgctatgcttcatgcgctatgacatactggagtatttcagcatctatgggacagcactgagcatgtgggtgtcattaatggcactggcagagttcgatgaaccaaaaaggtcaacctttgtaatgtttggcgtgttgactattgccgtgaggatctaccaagaccggtggggatatggggtatactcggggcctattggcacagctgtccttatcattgcaacaaaatggctgcaaaagatgaaagagaagaagggtctgtaccctgacaagagtgtgtacacccaacagataggccctggtttctgttttggagcgttagcactgatgctgcgtttctttttccaggagtgggattacacctatgttcacagcttctaccactgttcactagccatgtcctttgtcttgctgctgcccaaggtaaacaagaaagctgggaatgctgggacacctgccaaattggactgttctacactctgctgtgcttgcatctga

SEQ ID NO: 61 - DNA, 663 bp, synthetic construct
  misc_feature 1..663: note = Myomaker - Zebrafish cDNA
  source 1..663: mol_type = other DNA
atgggagcgtttatcgccaagatgttgctgcccactattagcagtttggtgtttgtgcctgcagccagcgtggctgcaaagaggggcttccacatggaggccatggtctatttcttcacaatgttcttcaccgcgatttaccacgcatgtgacggtccgggcttgtccattctctgtttcatgaagtatgacattctggagtacttcagcgtgtacgggacagccatctccatgtgggtcacgctactggcgcttggggatttcgatgagcccaaacgctcttcgctcaccatgtttggggtgttgaccgcagctgtgaggatttaccaggaccgactgggctacggcatttactccggccccatcgggacagctgtctttatgatcacagtcaaatggttacagaaaatgaaggaaaagaaaggcctttatccagacaaaagtgtttacactcaacaagtgggcccagggtgctgcttcggtgctcttgctttgatgcttcgcttctattttgaggagtgggactacgcttatgttcacagtttctaccacgtgtctctggccatgtcctttattctgctgctgcccaagaagaaccgttatgctggaacgggacgtaacgcagccaaactcaactgctacaccctctgctgctgtgtatga

SEQ ID NO: 62 - DNA, 10361 bp, synthetic construct
  misc_feature 1..10361: note = Myomaker - Human (+strand)
  source 1..10361: mol_type = other DNA
caagtgtgagctggggagggcaggggctcagagccgggctgggcgcagcatcagacacaagcacagcacagggtggagcagtccagcttggccggggtccccggggatccagccttcttgttgaccttgggcagcagcagaacaaaggacatagccagggcacagtggtagaagctgtggacataagtgtagtcccagtcctgcggggggcaagcggtcagtctggggcctcagccccctccccgaggctcctccctctccaagacccagcagagccccttcaggcccccgcctctgccagggcactgggacacctgcaggaagcctcccccacggtcgcgctcacagtggtttttctctccacctaaacccagagcagtgagggcctgtgccatcctccaggctgcactccttccttcttccccatcccctctctctgctgtccttctcttcctccatccttctctccctcctaccctccctccctccatctccccctcttttctctccttatccctcttcccctgttcctccctccctcctccactttctccctccttccttccctgtctcctcccctccctccctccctcctccaggtgttgggcacctgccccaggcgtctcccaggctgtgctgccgtctgagatgccagctgtctgtaggcagccagctttggtctctgtgacctccaggtccacacaggccatggtgctggtggtgctggggacggcattgcccccgacatagccctgggaggggctagtgagcagggactaataccagactttggcctggggctgtcagagtccccccagcgtgggcacagccctggtatcccagctgagcagagccatgccgagtgggctctggggcacaggacacctccccgctgggcttggtacctcaaagaagaagcgtagcatcagggccagcgccccgaagcagaggccggggcctatctgctgggtgtagacgctcttgtctgggtacaggcccttcttctccttcatcttctgtagctgtgaggacaggaggccacagcaaagcttttaggtcacagcactggggaacgcccctccccaaaccagcccgagagctggccctgcacaggctcaccccagccctctcccggcaggagaggaggctcaggagcctcctgccgcacccagcctcagatggcttctgctggacagggcccttcacggtgcgacccagcagagaccccagcctggatggctgggaaggaagccactgggccatgtgccccacaaagaccccgctgccctcccgcctctttgagatgtaacaacgccaccctcgcatgtctcctcctccctggaggggagctctggggggactagactccatgattgcttaccaaggaaagtactggagtacttgggacctgccagcccagtgtggcccatggggatggcacttgtggtgatccctgagccatggacaagcatcgtttgctttcctagttaaaggacctatctcactcttcattagacaaacttggccagcactgcttctcaggtcccagtgcttaggaaggctcgcgtgggcgtttccacttacagaggggtttgcattccgaggaagatgcgggaagtgtggggccacatccctggagccggccttgtgttttctaggccacttcacatggagtctatttgggattttcaagggcagttgtttcctggaatgagggtggatttttctccctgagcctggtcccctcttgggaggggctggggaacgacagccttgttggggaggaaggagggagggttgggtgatggcggcctcggagtggggccagacccgtgggggtacactcaggaggctatagatttcagtggaatcaactgttagacacacagcgtgtggcacaagcccctgggggtgggggcagcaccccataactgcacccattgctgagtggcctatgcaaagagcacaaagagccttatgctgggtcaggtcaggttttgccacccagtgaattatgaattgatgcccggctttccattttctggaattccattgccaacaaggaattgagcacctgcagtcctgcagtggcctgaagacagctggaccgtgtgaccctgggtgcggtggtcaaggctgccagcccacctctggccagccctgcagtagtaacaccagggagaagagaggtgcctgccccaggtcacacagtgggcctggcactattgaaagggcgccatcacccaaccctccctccttcttcctcccgggctgccattgcccaacccctcccaagaggggacgaggctcagggagaaaaatccaccctcattccaggaaacaattgcccttgaaaatcctaaataaactccatactaaatggtctagaagacaacaatttgagccccagatgcggggaggcgggcagcccatcctcggctcctgtggctggatctgcagcctgagggccttggcagtctcgtggctcttggtgggaaacacagcagtgaattctcttctgggcaattacagttcagcccagttcagacctggccaagaccagcgggaggagcaaccttcaggggcagaaggaggcgagaggcgggtggccaggacccagggccccagcacgctccttcctgccacccaccttggtccagcccacttatgcccagcgctccctctctccccaccaggtgactcccaggggcctcctgggtcagcccaggattagtgctgcttcctcaggttgcagacagaaagcaggtcctctgtctcctgctcaaaaagtcaagtccagccaggcgtggtggctcatgcctgtaattccagcactttgggagactgaggcaggcagattacctgaagtcaggagctcaggaccagccgggccaacgtggtgaaaccccatcgctactaaaaatataaaaattacctgggcgtgatggcatgcgcctataatcccagctactcgggaggctgagacaggagaatcgcttcaacccgggaggcggaggttgcagtgagccaagatggcgccattgcactccagcctgggtgacaagagcaaaactccgtctcaaaaaaaaaaaaaaaaaagtcaggttctggccccgccactgccctgccatgacgtcctgttaagttgctgaggcctccatgctttggttccttcataggccaaatggcaaatcagtcccatgctccttggctgtggggaggattgggacgggctttgcaagctgcccaccagaactcgagcgctctccccacagccgtgggccctcctgcactgagagctgccctctgtcttgctgggtgtcctgcggctctggccggggctggcagtgtggctgggctggaccaggccaggtcctctcttggcacttgaaactgaccctgagacttcaggtccactccaaagaggtgaaatgcagcacagggatgttcaggcggtgcctgggctgctgcaggcctggagagcaggctcaggctgaagcctgctggctccccaggtctgggagacccttgcaagggtgagctccctcctgctctggggtcccaggagatgccccgggtctatttttccctaagatccctctttagcttgggcgagtttgagtggggtttggtccctgagccaggagggtcttggtaggacggagagagcagggagcactgaagaccacgtgagggccttgctgctctgcaaggggctgtctgtgctagaaggtctggcccaggctgcctcactgtcataccacactctccctcctggctagaaccaagctcgaggctcactccctccaggaagtcttcccagattaccccaggccattttccaagttgatgttgcatctctaaagcagctggtagtaagagcggtgatgagagtgataacaaatagctcttatgtgcggagcacattggaagccaggctccatgccaggacttcaggtgcctgatctcagtgagtctttgaaccaccccatgagacaggcagggggctgtaatgacaacacctgctttacaggtacgggcgtggaggtgagacattgggtaacttgggctcagtctggagctggtgagtacagacaagcgtcacacacagtctacacagccggagcacctcatggctattttctacgtggttttgctgaattcctgcatccacccatttgcctatgagggcaggaggtaaatgaagatccgaggcaggaggagtcagacaggggagaggtgacgggcctcctgggtccccgttcatcgaggctcgcgcagtacgcacccactttgccgcgatgatgaggatggctgtgccgatggggcccgagtacaccccgtagccccatcggtcatggtagatccgcacagcaatggtcaggacgccgaacatcacaaatgttgacctcttgggttcgtcgaagtcggccagtgctggaggggccagggagacacagggggaggtgagtggtctctcttgctcctcctggctacccccccaccccccagcccccaggaggcatcctgtagatgccctctctcggtgtcccctcagccagcgagaccctgaggcccagcctggtcatggaggggtctgaattccagccagtttgagaggacaggcagcctgctgcttccccatggacacagcagcttggattgtgctcccagcacctcattttaataaacagaccacagctggttgtggtggctcaggtctgcaatcccagtgctttgggaggcagaggcaggaggatcgtctgagaccaggagttcaagactagcctgggcaacatagcgggacccccatctccacaaaaaattcggtgggtgtcgtggtgcatgcctgtcatcccagctacttgggaggctgaggtgggaggatggcttgaggctgtgagttcgaggctgcagtgagccgtgtttgtgccactgtactctggcctgagtgacagagtgagaccctgtggctaaaaatcaataatcactatgcaaagtgaataggatcgaatctatcccataggatcacaggacaaagacactaagattcaagagaagaaatgaagcccctcacaggcccggttagatggcaaggagcctcaggtcatggggaccttgccacagacaacagttacgtggaaaaaaacatggtgggaaagggggcttatgaacagtcccgtcttccaggctggatatcacccgtgtgtgtggatgtttgtatgacagtctgggaagccaacccccctgagcagtgaacagcggtcctcccagggaaggagtgacgggagggagccctttcactttttcctttgtatgcctctgctgttgaaatgtgtcacaacaagcttttactaaatgagtcattttaaaaggatataaaaaatcggcatcagggcatttaagaggtgcatattctttttcatagattaagcacaaccctgaaacccagacaagggaagacattcctggggctgggagtgagtggggatagagggctgcagcgggactggtttgaggctgggtgtgcggacactggggagccggtccttgtccgcaaggcttgtctgcaggggttgaccactcacccatcagcgagacccacatgctcagggctgtcccgtagacactgaaatactccaggatgtcgtgacgcatgaagcacagcacagacaagccgggtccattgcaggcatggtggagctgccagaaaacccacaggtggtcacagcacaaagaggccagagctggtccccgagccacggcccccagagtgccaggtcacttgctggctgtgagaagtcactttggcgagtcacttaatgactgtgtgcctcagtctccccgtctgaaaaatgggggtactgccgagcactcccgcagagggtcctgtggggattaagtggcacatgccagcgaggtgtttaggggctggggtgtgccaagggttcactcaatgtcacctcagcagaattcgctcatctgcactggcaggactgggcggagactgagtggtcactcaggtgaagcccgcttaggtggggcggtctccgggagggaccctacacggctctccccggaccttcagcatctgtgcttccttgaagcacacagctgcgtgttcactcgccaatctttggatgtgaggtcagagcctctctgggggctcctttgctctttgggggctcctggggccttctcttgcacaaattacccctctgatgactggtctacactgcagcagcgttctcaggcttgagtgggcatcagaacgcctggggccttgtttagacacaggttactgagccctgcctagggttgctgattagggagggctgggttgggtagaaaatgtgcattttgaacacattccctgtggcactgctgaggctggcagggcccacactgagagccgggctgtagctcctggtttctgttgccttaacgtggacgaagatctctgagacccccttgcagaagctgaacacagccccctaggctcatccatctctgccctatactctcgtcgtcgcctccccaacacccactttcatggcaatttttaaggcaaaaggcttatagggagtgttttcaaagcagtcaactacttttctacggaaaacaactctctctccttttgcattcgcatttcatcattttaggtaatatttaattacatgacataattattttgacaggttcaactggcacaaacaagcttgggaaacagcacggtggactcttggtcagcccagctcagcgggaggagcaggcgtgctggaaagcagcccgtgtctggaggcgacagggacagcacagagggagcgggggccctgggtgatctggggggcaggcaattcggggtcaaagtggagtgcttctactgatggcaattgtacacggcctaaagtgacggtgcacctaggaggcattaatagggatccagcatctaaaatgagggaggcggcggtcctgcttctctctgttcttgtcaggctcatccagaagactatgccgagctctgtgtggtgcacctttcttgaagtgagactgggaaagacgcggctagaggagggtgaccagcggtggacatgactgtttaccttggggacagggaagcttcaggaggggcctgatcaaggtgcttacacctctgtgggaaagaggagcgaggaagactccggccctaggctgttctcctgttctcctggcttcttcccatcccccaccccagccccatcacctgctgtctgtgtgcctcaatgtagcacagatggtcatgtgtgattaaggcattcactgtgagattgtgataaggcctgtgcccttgccctgccaggagcaggaatggctctgtctggtcccagttgcatggacggctcccagcatagagtgcttgctgcatgtgttcagggagggggacgccaggctctgagaattctaaaggacagccagctcaccctggggacccagagcctctgccactaggcccttggctcctcccaatggtgggaacttagctccattcgacagatggggaaagtgaacttcagagcagcactgcctgcccaaagaggtgaaacagagcagtgcttggcacctggccacttcctcccatcctgcagtgcagggggcagacctggcccagccggggcactggtggggtgggtgcggctgagggcctggggggtcagagctcaggctcggggagtctgactttgcagatgttcccagtgggggctcaggtgagtggctgtcgggggggggcctcctctgttgtgtggggacaagcacactgtctccgtggggtttgcacccatagcaaggtgtccggcacagagatggagattgtcacgggaggggcctgattggaagggaagggacgccatgcgggtggcagaactttgggagggactgagtgtggctttgagttcagaagacgtttgtcacaagaggcagctgcccctgccactctgggtggggcagggtggggcctctgagaccagtgcagaggcagctgcggggccagcctaggcccaggcagggaggtgtggcctggtgggtgcttgtggtttgctgggctaggtctaacaggagccttgagaacaagacctcagcttttctccctgcgctaaggccatgggacctgcagagaaatcctggctctgctctgggcttcagtctctcatctgcccaagaggcttcctagccctagcccaggctggagtcccagaggagcgaatgcagtggcatttgggtgagtcaggagctctggagagcttgatggtcacagtgacacaagtgactctgtctctctgggatttggtttcttcatctgccaaatgggaatcaagatcctaggcttgtggggaaggtgaaaaggctgaatcagacactgtgcacagagcgcctagccgagtcctctgccctgggtactggcgctcgaggtggactcagaagctccagggcatctggttccacaaaggacccagcctgtcccaggccactgtcacccctgggagtggcacacactggagggaatgcctcgctcccagcccacacgtgcacactcagcttctgccattgcgggcaaaattggacttgaccaattcaggatacaagcataacatgtgaatatatgcttgcaaacacacgtgtgagctcacgggcctcacccgctcaggactccctctgtgcactcacatgcacttggcattcttgcccatagaggccctgctgctggagaaggaggctgtctggggagaggaggtggagttttcacaggttgggcccagcactgccccaagaaggaggctagtgggacgcttgcctccccagagcaggtgtcatgctggggattgggctgtcagtgaaggaggggtgtgatggaaggtgagcaaggaaggcttcgggagagcaagaggtggggcaccacttgtgggagtccaggagtgagggcatgttagtggagaaagtcggaaagacccagaggcaagaaggcagggggtaccgagacatataaatgatggctgaatggcgagatggtaatagacgaatagatcacaggtagatggatgcgtagatagagagatagatggagagagagagagagagagagagagagagagagagagacaagctggagaaggtggatagctaaagccagagagacacatggagagtcaggggactaaaaccagggagggtgggaccaagagctttagagagagtgaattccatggggatcgagttccagaaatcaaaagagaaccagacagagagagaaaggaaaaaaagagaaacagagaaaactagacacagaaaaccaatacgagaaacacagagtgaaagagacccagaaagagagagagagaagacaggggagacaggggtcccagaaacagcgacctcagaaacaaggacagatggggttctgggcgctccactgaaagccggataagatcacccaatgacaggtaccaggaaacagagagcaggagagagccagagagagagcaagcggagacagtcagccagccagacacataaatagaaagagaaagacggacccacagagagagaagtaggccccagaagagggagagaccagcaggccctcctgaaccagagcagctccaggattctggaatcagactcactcacccaggccttcacactccctgaaccctgcagaccccttcccaggcctggcttgccccactcatctctgctccatcgtggcctatgggtagagctcgaagagaggtggggaggggaggtggccccatgggcagccgtgggggctttgattagcagctgagaaaaggggcacgctggaagggtttatcctcaactcaatggccctgcttcaccccaggcttggtctcacacaggcagtgatcccagagcaacttcctggcacagatgggaaaactgaggtccagataggggaagggactcccctagtcctctctcttcagtctccagaccccacctgggcctgctgtttcattttcaaatcacttctgctcatcacccaatacaagaacgctgtggacagagagcctctcctctacctccaggatggggcctgtgtgggacttcctcccagcccccagactcaccgccacgaagaacagggtgaagaggtagaccatggcctccatgtggaaccgcctcttggccgcgatgctgacagtggggaggaaggccaggctgctgagggtgggcaggagcagcttggccaccagcgtccccatgggccaggaggaaagcactggctggggtggggagggtgctggtgtcccaggtccccagcacaggagcacgaagtgggaaggccagctccctttgggcagggc

SEQ ID NO: 63 - DNA, 10361 bp, synthetic construct
  misc_feature 1..10361: note = Myomaker - Human (-strand, reverse complement)
  source 1..10361: mol_type = other DNA
gccctgcccaaagggagctggccttcccacttcgtgctcctgtgctggggacctgggacaccagcaccctccccaccccagccagtgctttcctcctggcccatggggacgctggtggccaagctgctcctgcccaccctcagcagcctggccttcctccccactgtcagcatcgcggccaagaggcggttccacatggaggccatggtctacctcttcaccctgttcttcgtggcggtgagtctgggggctgggaggaagtcccacacaggccccatcctggaggtagaggagaggctctctgtccacagcgttcttgtattgggtgatgagcagaagtgatttgaaaatgaaacagcaggcccaggtggggtctggagactgaagagagaggactaggggagtcccttcccctatctggacctcagttttcccatctgtgccaggaagttgctctgggatcactgcctgtgtgagaccaagcctggggtgaagcagggccattgagttgaggataaacccttccagcgtgccccttttctcagctgctaatcaaagcccccacggctgcccatggggccacctcccctccccacctctcttcgagctctacccataggccacgatggagcagagatgagtggggcaagccaggcctgggaaggggtctgcagggttcagggagtgtgaaggcctgggtgagtgagtctgattccagaatcctggagctgctctggttcaggagggcctgctggtctctccctcttctggggcctacttctctctctgtgggtccgtctttctctttctatttatgtgtctggctggctgactgtctccgcttgctctctctctggctctctcctgctctctgtttcctggtacctgtcattgggtgatcttatccggctttcagtggagcgcccagaaccccatctgtccttgtttctgaggtcgctgtttctgggacccctgtctcccctgtcttctctctctctctttctgggtctctttcactctgtgtttctcgtattggttttctgtgtctagttttctctgtttctctttttttcctttctctctctgtctggttctcttttgatttctggaactcgatccccatggaattcactctctctaaagctcttggtcccaccctccctggttttagtcccctgactctccatgtgtctctctggctttagctatccaccttctccagcttgtctctctctctctctctctctctctctctctctctctccatctatctctctatctacgcatccatctacctgtgatctattcgtctattaccatctcgccattcagccatcatttatatgtctcggtaccccctgccttcttgcctctgggtctttccgactttctccactaacatgccctcactcctggactcccacaagtggtgccccacctcttgctctcccgaagccttccttgctcaccttccatcacacccctccttcactgacagcccaatccccagcatgacacctgctctggggaggcaagcgtcccactagcctccttcttggggcagtgctgggcccaacctgtgaaaactccacctcctctccccagacagcctccttctccagcagcagggcctctatgggcaagaatgccaagtgcatgtgagtgcacagagggagtcctgagcgggtgaggcccgtgagctcacacgtgtgtttgcaagcatatattcacatgttatgcttgtatcctgaattggtcaagtccaattttgcccgcaatggcagaagctgagtgtgcacgtgtgggctgggagcgaggcattccctccagtgtgtgccactcccaggggtgacagtggcctgggacaggctgggtcctttgtggaaccagatgccctggagcttctgagtccacctcgagcgccagtacccagggcagaggactcggctaggcgctctgtgcacagtgtctgattcagccttttcaccttccccacaagcctaggatcttgattcccatttggcagatgaagaaaccaaatcccagagagacagagtcacttgtgtcactgtgaccatcaagctctccagagctcctgactcacccaaatgccactgcattcgctcctctgggactccagcctgggctagggctaggaagcctcttgggcagatgagagactgaagcccagagcagagccaggatttctctgcaggtcccatggccttagcgcagggagaaaagctgaggtcttgttctcaaggctcctgttagacctagcccagcaaaccacaagcacccaccaggccacacctccctgcctgggcctaggctggccccgcagctgcctctgcactggtctcagaggccccaccctgccccacccagagtggcaggggcagctgcctcttgtgacaaacgtcttctgaactcaaagccacactcagtccctcccaaagttctgccacccgcatggcgtcccttcccttccaatcaggcccctcccgtgacaatctccatctctgtgccggacaccttgctatgggtgcaaaccccacggagacagtgtgcttgtccccacacaacagaggaggcccccccccgacagccactcacctgagcccccactgggaacatctgcaaagtcagactccccgagcctgagctctgaccccccaggccctcagccgcacccaccccaccagtgccccggctgggccaggtctgccccctgcactgcaggatgggaggaagtggccaggtgccaagcactgctctgtttcacctctttgggcaggcagtgctgctctgaagttcactttccccatctgtcgaatggagctaagttcccaccattgggaggagccaagggcctagtggcagaggctctgggtccccagggtgagctggctgtcctttagaattctcagagcctggcgtccccctccctgaacacatgcagcaagcactctatgctgggagccgtccatgcaactgggaccagacagagccattcctgctcctggcagggcaagggcacaggccttatcacaatctcacagtgaatgccttaatcacacatgaccatctgtgctacattgaggcacacagacagcaggtgatggggctggggtgggggatgggaagaagccaggagaacaggagaacagcctagggccggagtcttcctcgctcctctttcccacagaggtgtaagcaccttgatcaggcccctcctgaagcttccctgtccccaaggtaaacagtcatgtccaccgctggtcaccctcctctagccgcgtctttcccagtctcacttcaagaaaggtgcaccacacagagctcggcatagtcttctggatgagcctgacaagaacagagagaagcaggaccgccgcctccctcattttagatgctggatccctattaatgcctcctaggtgcaccgtcactttaggccgtgtacaattgccatcagtagaagcactccactttgaccccgaattgcctgccccccagatcacccagggcccccgctccctctgtgctgtccctgtcgcctccagacacgggctgctttccagcacgcctgctcctcccgctgagctgggctgaccaagagtccaccgtgctgtttcccaagcttgtttgtgccagttgaacctgtcaaaataattatgtcatgtaattaaatattacctaaaatgatgaaatgcgaatgcaaaaggagagagagttgttttccgtagaaaagtagttgactgctttgaaaacactccctataagccttttgccttaaaaattgccatgaaagtgggtgttggggaggcgacgacgagagtatagggcagagatggatgagcctagggggctgtgttcagcttctgcaagggggtctcagagatcttcgtccacgttaaggcaacagaaaccaggagctacagcccggctctcagtgtgggccctgccagcctcagcagtgccacagggaatgtgttcaaaatgcacattttctacccaacccagccctccctaatcagcaaccctaggcagggctcagtaacctgtgtctaaacaaggccccaggcgttctgatgcccactcaagcctgagaacgctgctgcagtgtagaccagtcatcagaggggtaatttgtgcaagagaaggccccaggagcccccaaagagcaaaggagcccccagagaggctctgacctcacatccaaagattggcgagtgaacacgcagctgtgtgcttcaaggaagcacagatgctgaaggtccggggagagccgtgtagggtccctcccggagaccgccccacctaagcgggcttcacctgagtgaccactcagtctccgcccagtcctgccagtgcagatgagcgaattctgctgaggtgacattgagtgaacccttggcacaccccagcccctaaacacctcgctggcatgtgccacttaatccccacaggaccctctgcgggagtgctcggcagtacccccatttttcagacggggagactgaggcacacagtcattaagtgactcgccaaagtgacttctcacagccagcaagtgacctggcactctgggggccgtggctcggggaccagctctggcctctttgtgctgtgaccacctgtgggttttctggcagctccaccatgcctgcaatggacccggcttgtctgtgctgtgcttcatgcgtcacgacatcctggagtatttcagtgtctacgggacagccctgagcatgtgggtctcgctgatgggtgagtggtcaacccctgcagacaagccttgcggacaaggaccggctccccagtgtccgcacacccagcctcaaaccagtcccgctgcagccctctatccccactcactcccagccccaggaatgtcttcccttgtctgggtttcagggttgtgcttaatctatgaaaaagaatatgcacctcttaaatgccctgatgccgattttttatatccttttaaaatgactcatttagtaaaagcttgttgtgacacatttcaacagcagaggcatacaaaggaaaaagtgaaagggctccctcccgtcactccttccctgggaggaccgctgttcactgctcaggggggttggcttcccagactgtcatacaaacatccacacacacgggtgatatccagcctggaagacgggactgttcataagccccctttcccaccatgtttttttccacgtaactgttgtctgtggcaaggtccccatgacctgaggctccttgccatctaaccgggcctgtgaggggcttcatttcttctcttgaatcttagtgtctttgtcctgtgatcctatgggatagattcgatcctattcactttgcatagtgattattgatttttagccacagggtctcactctgtcactcaggccagagtacagtggcacaaacacggctcactgcagcctcgaactcacagcctcaagccatcctcccacctcagcctcccaagtagctgggatgacaggcatgcaccacgacacccaccgaattttttgtggagatgggggtcccgctatgttgcccaggctagtcttgaactcctggtctcagacgatcctcctgcctctgcctcccaaagcactgggattgcagacctgagccaccacaaccagctgtggtctgtttattaaaatgaggtgctgggagcacaatccaagctgctgtgtccatggggaagcagcaggctgcctgtcctctcaaactggctggaattcagacccctccatgaccaggctgggcctcagggtctcgctggctgaggggacaccgagagagggcatctacaggatgcctcctgggggctggggggtgggggggtagccaggaggagcaagagagaccactcacctccccctgtgtctccctggcccctccagcactggccgacttcgacgaacccaagaggtcaacatttgtgatgttcggcgtcctgaccattgctgtgcggatctaccatgaccgatggggctacggggtgtactcgggccccatcggcacagccatcctcatcatcgcggcaaagtgggtgcgtactgcgcgagcctcgatgaacggggacccaggaggcccgtcacctctcccctgtctgactcctcctgcctcggatcttcatttacctcctgccctcataggcaaatgggtggatgcaggaattcagcaaaaccacgtagaaaatagccatgaggtgctccggctgtgtagactgtgtgtgacgcttgtctgtactcaccagctccagactgagcccaagttacccaatgtctcacctccacgcccgtacctgtaaagcaggtgttgtcattacagccccctgcctgtctcatggggtggttcaaagactcactgagatcaggcacctgaagtcctggcatggagcctggcttccaatgtgctccgcacataagagctatttgttatcactctcatcaccgctcttactaccagctgctttagagatgcaacatcaacttggaaaatggcctggggtaatctgggaagacttcctggagggagtgagcctcgagcttggttctagccaggagggagagtgtggtatgacagtgaggcagcctgggccagaccttctagcacagacagccccttgcagagcagcaaggccctcacgtggtcttcagtgctccctgctctctccgtcctaccaagaccctcctggctcagggaccaaaccccactcaaactcgcccaagctaaagagggatcttagggaaaaatagacccggggcatctcctgggaccccagagcaggagggagctcacccttgcaagggtctcccagacctggggagccagcaggcttcagcctgagcctgctctccaggcctgcagcagcccaggcaccgcctgaacatccctgtgctgcatttcacctctttggagtggacctgaagtctcagggtcagtttcaagtgccaagagaggacctggcctggtccagcccagccacactgccagccccggccagagccgcaggacacccagcaagacagagggcagctctcagtgcaggagggcccacggctgtggggagagcgctcgagttctggtgggcagcttgcaaagcccgtcccaatcctccccacagccaaggagcatgggactgatttgccatttggcctatgaaggaaccaaagcatggaggcctcagcaacttaacaggacgtcatggcagggcagtggcggggccagaacctgacttttttttttttttttttgagacggagttttgctcttgtcacccaggctggagtgcaatggcgccatcttggctcactgcaacctccgcctcccgggttgaagcgattctcctgtctcagcctcccgagtagctgggattataggcgcatgccatcacgcccaggtaatttttatatttttagtagcgatggggtttcaccacgttggcccggctggtcctgagctcctgacttcaggtaatctgcctgcctcagtctcccaaagtgctggaattacaggcatgagccaccacgcctggctggacttgactttttgagcaggagacagaggacctgctttctgtctgcaacctgaggaagcagcactaatcctgggctgacccaggaggcccctgggagtcacctggtggggagagagggagcgctgggcataagtgggctggaccaaggtgggtggcaggaaggagcgtgctggggccctgggtcctggccacccgcctctcgcctccttctgcccctgaaggttgctcctcccgctggtcttggccaggtctgaactgggctgaactgtaattgcccagaagagaattcactgctgtgtttcccaccaagagccacgagactgccaaggccctcaggctgcagatccagccacaggagccgaggatgggctgcccgcctccccgcatctggggctcaaattgttgtcttctagaccatttagtatggagtttatttaggattttcaagggcaattgtttcctggaatgagggtggatttttctccctgagcctcgtcccctcttgggaggggttgggcaatggcagcccgggaggaagaaggagggagggttgggtgatggcgccctttcaatagtgccaggcccactgtgtgacctggggcaggcacctctcttctccctggtgttactactgcagggctggccagaggtgggctggcagccttgaccaccgcacccagggtcacacggtccagctgtcttcaggccactgcaggactgcaggtgctcaattccttgttggcaatggaattccagaaaatggaaagccgggcatcaattcataattcactgggtggcaaaacctgacctgacccagcataaggctctttgtgctctttgcataggccactcagcaatgggtgcagttatggggtgctgcccccacccccaggggcttgtgccacacgctgtgtgtctaacagttgattccactgaaatctatagcctcctgagtgtacccccacgggtctggccccactccgaggccgccatcacccaaccctccctccttcctccccaacaaggctgtcgttccccagcccctcccaagaggggaccaggctcagggagaaaaatccaccctcattccaggaaacaactgcccttgaaaatcccaaatagactccatgtgaagtggcctagaaaacacaaggccggctccagggatgtggccccacacttcccgcatcttcctcggaatgcaaacccctctgtaagtggaaacgcccacgcgagccttcctaagcactgggacctgagaagcagtgctggccaagtttgtctaatgaagagtgagataggtcctttaactaggaaagcaaacgatgcttgtccatggctcagggatcaccacaagtgccatccccatgggccacactgggctggcaggtcccaagtactccagtactttccttggtaagcaatcatggagtctagtccccccagagctcccctccagggaggaggagacatgcgagggtggcgttgttacatctcaaagaggcgggagggcagcggggtctttgtggggcacatggcccagtggcttccttcccagccatccaggctggggtctctgctgggtcgcaccgtgaagggccctgtccagcagaagccatctgaggctgggtgcggcaggaggctcctgagcctcctctcctgccgggagagggctggggtgagcctgtgcagggccagctctcgggctggtttggggaggggcgttccccagtgctgtgacctaaaagctttgctgtggcctcctgtcctcacagctacagaagatgaaggagaagaagggcctgtacccagacaagagcgtctacacccagcagataggccccggcctctgcttcggggcgctggccctgatgctacgcttcttctttgaggtaccaagcccagcggggaggtgtcctgtgccccagagcccactcggcatggctctgctcagctgggataccagggctgtgcccacgctggggggactctgacagccccaggccaaagtctggtattagtccctgctcactagcccctcccagggctatgtcgggggcaatgccgtccccagcaccaccagcaccatggcctgtgtggacctggaggtcacagagaccaaagctggctgcctacagacagctggcatctcagacggcagcacagcctgggagacgcctggggcaggtgcccaacacctggaggagggagggagggaggggaggagacagggaaggaaggagggagaaagtggaggagggagggaggaacaggggaagagggataaggagagaaaagagggggagatggagggagggagggtaggagggagagaaggatggaggaagagaaggacagcagagagaggggatggggaagaaggaaggagtgcagcctggaggatggcacaggccctcactgctctgggtttaggtggagagaaaaaccactgtgagcgcgaccgtgggggaggcttcctgcaggtgtcccagtgccctggcagaggcgggggcctgaaggggctctgctgggtcttggagagggaggagcctcggggagggggctgaggccccagactgaccgcttgccccccgcaggactgggactacacttatgtccacagcttctaccactgtgccctggctatgtcctttgttctgctgctgcccaaggtcaacaagaaggctggatccccggggaccccggccaagctggactgctccaccctgtgctgtgcttgtgtctgatgctgcgcccagcccggctctgagcccctgccctccccagctcacacttg

SEQ ID NO: 64 - DNA, 10526 bp, synthetic construct
  misc_feature 1..10526: note = Myomaker - Mouse (+strand)
  source 1..10526: mol_type = other DNA
ttccaggaactagaatgtatgttaggcgaagctaatgactagtggctgatcaagagtttactgtgaatggcttgatcgaaaacctgcagaagggatgggactcaggcaggggtatgcaaggttcgctggctccagcttcctaagtggagagctttcagagcctgggcaggggttaaaagggcaatcccagtttcctagggaaagcagacgattctgacaggcaggacctgggaaatagataaccctgcatgctgctgggtatttactggtctagggttctctgccaggcacacctatggttgtgaggccttgggggataaagttcttttttttcctgaacagagtgaagcaactggtgaacacagaaccagtgggtccctaagcagcactcagcagaatgcagcaggcctgctggtctcttggggtgtagagaagaccatttctcatgtacaggccgcataacaaagtataggaagtaccttgggagagacagcaggactgccaggcaggaaggcaggggcctggtgtgtgtgtgtgtgtgggggggtatagtcagacacaagtgcagcagagggtggagaaggtcagcttggcgggggcccctgcgttcccagccttcttgttgaccttgggcagcagcaggacaaaggacatggccagggcacagtggtagaagctgtggacgtaggtgtaatcccattcctgtggaggagaatgagtcagtctgggcctccatcccttccctaaaccaagtcctagccatttggtgcctctgtcagccagcccaccctgagaaggtggcagaaaggcttgctgccttcctctgttccatgcctcctgggtgctgggcaccagctcctggttccttccaggacatgcgtgcatcttgggtgcaggcttcctaaagtcagggcctgacttgtccactcaggcagtgaggctagtacactggggatggtgagtaccatcctcaagaggacagaatttacaacttggagcctccatatgtggctgttagttaactatttccagaggctcttgctccccttccccataggccaggtacctcaaagaagaatcgaagcatcagggccagggccccaaagcacaggccggggcctatctgctgggtgtagatgctcttgtcggggtacaggcccttcttctctttcatcttcttcagctgcaggcacaaggtggggacatcaaagttcttggggtgcagcacaggaagggacccctccatgaactgtagaagagccctacccccattcctctgtatgcctgactgatgggactctctgggccaatttcccctgggtcctctactgcccgcatctggtgggctttggcacttcagtggcagacgtgatcagttttcccagctaaggggttttcctctgttaaccttggtttcataggccctgtgtgttcaagcttggtaagatggagtgttacatggaatagatgggagtcccatggttcctcactggaatgcacatccttggggcccaaaggtattttaggtattcaagattgttcaggtttcagtggggaagatcattataaataccactgtcaggtgtgcacagagggcacaggacagcagccctgactgagtgatgtgcacagtgggcacaggacagcggccctaattgcacacctcactaaatacattatatgtacaaatgctgtcaatggcctcgtgcaaatcagggcaagctttgtcactctgagtgatgatatgttgctgtttccaagtgttctaaaacttgccattagtaacaggagtggaggtcccagtgagcagtgccagtgacatgggcaccgcctattagcctgagtgtaggccgtatgaccatcaatcacacagttctaacactggggccccagagaggagaagaatattgaagatcacccatgggccctgtcttgccccgggaacccctatttcccatttcactcagcttcttctccccaaatgttgtattcatgttcctttcctgaaagggtgagacatgggaaagaattgtactccgttctaagaagtaagtccaaaccacctgcctatctaagatctaggagatggggtctgtgccccaggcatgggtggctgcagcccctcactcccattctcaccagagacctggggaggctggcatttagtggaggggggcactggcacatgtatgctatcctggctaattaaaatcccatcaggatgggtgtgctgggcttggacaccagcattcaagaggcagaggcgggcagatctctatgagtttgaagccatccagagatacaaagtgagagtctatctttaaaaacaaacaaacaaacaaacaaacaaacaaacaatcaagtcagatccagaaccagtgaagagcagcaaggggccatgataggcaagacaaagaggcagttatcagagcaagccttcttgtttatgcattccagcttgttaactagccatgcagaagcccaacacctctgccttgggtcagagagggccagcttcggctcctcaaactggagtgggatggaagcttctcccctcgaaagtcaagcacagctgccattacctactagggctgcaggttaggctgctgagctctgtgcatttcaggttcatccttaacttaaaatcagaataagcccgggttcctcggagcccacaggagtaggatgtggcttggaagcttcctccctgactatacctgtccccactttgctgaagatggatcagagctctcccacccctggccctgccactcccctctgacacagacacagacacagacacagacacagacacagacacagacacagacacagacacagacacagacacagacacagacacagacagacacagacacagacagacacagacacagacacagacacagacacagacacagacacagacacagacacagacacagacacagacacagacacacaggcatagacacagacacagacagacacagacacagacacagacacagacacagacacagacacagacacagacacagacacagacacagacacagacacagacgacacagacacagacagacacagacacagacagacacagacacagacagacacagacacagacacagacacagacgacacagacacagacagacacagacacagacacagacacagacgacacagacacagacagacacagacacagacacagacacagacacagacacagacacagacacagacacagacacagatgacacagacacagacgacacagacacagtcacagacacagacacagacgacacagacacagacagacacagacacagacagacacagacacagacgacacagacacagacacagacacagacgacacagacacagacagacacagacacagacacagacagacacagacacagacagacacagacacagacacagacacagacacagacacagacgacacagacacagacagacacagacacagacacagacacagacatagacacagacacagagacacagacacagacaacacagacacagacacagacacagacacagacacagactcagacacagacacagacacagacacagacacagacacagactcagactcagactcagactcagactcagactcagactcagactcagactcagacacacagtcacacagacacacacagacacacacagacacacacacaaaggcacacacacacacaaaggcacacacacacacacacaccccaccgcctgccccaatctgcactgctgtagctctacttccaggaacctgcaagatcccaaatggtgcttcctgcatgaggtagcagacaggtgagaacttgaagcctgagtgctgtctgcttggtctgaagcctgctggcctggaaggtctgtgttttgggcctaactgctctgggtggagctcagaaaacatccctgggtctttcctgctattgggaaatttgttcacgatggctaacttaggtgggttttaggccatggaggtgagagggccttgagaccatagaggggttaggagcctatacagcagagtagatgccaagcgccaggccctcctctaggcctcccactcaataccctgcttcacccccacctcacaccttccttcctcatgagaaccatttccaaggcttgcttctttcgggaagactatccagattaacctatctgctctccaaactggtattatacctgtaagcagtgttgtctctcagaatgataatgatagtgatcttatgttgatgaaaagactgacagtgacagtcatgatgacaaaaggtctcctcagctctgggtatattaaaaatcacacctgtgcctgtgcctgtgcttagaagcattctttatgggtatttggatgcagagcagaggtcaagagaaaaggagttttggctttatccaggaccaataaaccagcagggcatgggacccgagcatgagccaccatttttaggaattttagggtttttggcccaattcttactaattcacctgcatataaggatatggggtataggaccctacataggagaaaccaagatcagggaagaaatgcaggttccgtggtctccgacagtggagatactggaagtactcacccactttacagcaatgatgagggtggccgtgcctatgggaccggagtataccccgtaaccccagcggtcatgaaaagtccgcacagcgatggtaaggacgccaagcattgtgaaggtcgatctctggggttcatcaaagtcggccagtgctggggagaggcatagctatggtgagcagcgtccctcacatggctgtgcctccatccttgggaacctattggtatgtcctctcaatctgtagggccagcctggtttccataaggtctgaattttggttatttggagggagtgggtgatgctgcttccctggagcagggtggctgaaataaactggtagactgagtgaccagcatttcctaggaatcctgagacaaaagtgttaagactaatgattggtgcgcagagctgagtctcaggagggaccccgggactgcatccctgggagacaagggtgagcttgcttggtttctcccttttctctttccttcccttccctttctttcccctttctttgctctctccctccttctctccctgtctcccttcctccctccctccctgtctcctttcctttcttcttccttcatcctttctgctttctacttttctctatctcttccttctttttctttcaaaattttgcagttgctggtaatggaatgaagggcctattgattaccaggcgagcgatctgccattgagctgtatataccccaggtccaaggtgaggattttgaatggtctgccttcctaatacacagagctgagctgacccatgagggcaaatgctcctctgagcctggaggacaagctgggaggctaggtccaggatgcctttggcctctcctttgtatgcttctgttttttaaatgtcacaagtgctaactactggagtcacttaaggatggtggaaatgagagtgcaggcatcagagaaatgtgcatgtctctttaagcagattaagctctgcaaagcagcaaggagggaggatctcagagaggggctgggtactggctggggttcaggactggctcccacccattggccaagatggccacttacccatcagggagacccacatgctcagggctgttccatagatgctgaagtactccagaatgtcacggcgcatgaagcacagcacagacaaaccaggcccatcacaggcatgggagaactgtagggaaatcacatgaggtcagcaggcagtgggcagcccaggagtgggtgagaactggtcccaaggctcaggttcactagctgtgagcccctaatggttttgtacctcagcctcctccctcacactatcagagcccttgtggagattaaacaggtgagtccatctagcctgggagtgcaaaagtctttgtaaatatccctttcagactcagcactggcccaaggctggtgagaagcatgctcagaagggcatccttaaagaccacttacacctttgcccatgactgactgaaagtgtacacattcctatgccagtctttgcataggagccttttatcctggacccctgtctctccataaaagaggaagcccttagattccccccaagcaagtgctgattctgacacactggtttctttcccccatatgccagcaggtgtgtccctgactcgtagttgaatagatttgcttctaagcaaaaggttctatatgcaggatttccaagcagacaacttatttcttgcagaaaacaacttgctctccctttgcttcacatttcatcattttaagtaatatttaattacatgacataattattttgacaagtgcaactggcacaaacaagcccagcagccagcacaatgagctcttggtaagcccaacttagcaggagggagcaggcaagctggaaaacagccttgtctggaggcagcaggggcaccaccgagggaggcaggcggagagctggggaccctggatgatggatgtatcagtcaagcacatagggcctacttagaagctcagagacctcctgctggtcacagttgcacatggactctgtcaatcaatagagagcatccaggggaagggaggaggtggtccagcctctgtgttgggtcagccccagccttgagctttgggttctgcaccttttaaaagggagattggtgaagaggaggttaaccaactaggtatgagctcaggaaaagacaagctttgggttgggccagaccaaggtacgcaagtggagaaggaaaggaactcagctctgggaggggactctgctcttctggctccttacagaaccacatgaccccaccccaccccacctgagcccatcatctgtagcatcttgcttccttctcttgtataggcccccatgaatgagtaaaacttacttactgtgagatcctgggaaacactcatgccttcccccacgaggagaagagcttccttaggcttgatctcaacatagaatacttggctacatgtgaaggccagaggagcaggctttctaacaagggatctaactgtcctcaggccctgaggattaattttttggggggtgggtgacctgtgtgacagtgaacttccctggggaacctcctgcccaaggaggcaggggcaaggctgtgatgtgtaccctttctccccagaggcagggagatctggtccagctggtgccaggctaggacacagctgggtgtgacaggagccctaaccctgctgtcagctcagagctggcagaggggcccaggttctctcaggtctctcaggcccaccttgtctaatggcatgagaacacctgttctgtggggcttacaaggggaccctaacgataactgcggagcatggcaccccacactgcaaaaatgaaatgctgtttaaagtttgctttcattaatcaaactttcccccaacctgaaaccaagttaatatgtgcgttatgggcatttaaacaatgtgcttgccctgggcagaattagctcacctctgggaaaaacaattcaatcgatcttattatgctttgcatttctggtggaggactctagtgagtctttgtgactctttcatgcccgactcagaacagtatatgtttgtgtgagatgtggtgaccaggtctaagaccacgtgtgttagaaacagcaaggtatggagaccatgttgaaagcaaaatgtgggtgtaggctgataatatctgattgtggatttgtgtgctactgagtcaaagggccagagagacagctgtctgctataaaagcctaagactcagatcccattctttttgtccctgtttgttgtgctgttcagcaagtagaaaggatgatattgtctaagattcttagattagaacctgattttagattagatgactatcaggttagaacaggagagggcagaattctttggaatacatcagatccacccgctgtgtaactgacaccaagagtcattcttctattcagcagcagcataccatacaactggtagttgtcatggagagtcctacagcagccacgtggaaggcagaactctgtgaggaacagattgtggctttgaggccagaggacatttgtcataagagacagctggccctgccactctgggtggggtgtggcagggtgggcctccaaggccagtgcagaggcagctgtaggccaattagacccaggcaggcaggggtgacctgattggggctgtgatttgctggactgtatctaacacaggccttgggaacaagaccctggcttatgtccttgaccgtggggtctcatcttggctctgaccttggccaggtctcaagaggaacaaatgacagtgtgggacaaagtactgtggggcagaccaggatctgagtgttcatggtgacactggtggcccagtttctctgagactcagtttcctcttctatcaaattgaaatcactatgttaggctcgtgggtgataatgagtccaaccccaccatggttgctttcttgtgacttatcattggcctaatgtcctcccctactgaagtgaactcaagagccatagagtttccagttccttgggttacctatgggaccaccacaaccaggaggtagacaggtgccaagccctcccccactgttctcagcccacatgcattgtggcttctcccaccactagaaagtcatgccagctgactcaggatatggaacacgcatgtgagcacagatgtgtgagtttgtgggctcactcattgagagccagctggataccttcacatactctatgcccttgccttactgagacctgctgcaggaagggcaggcctaaggagaggatgctagtctctaaaagtttggctctgctctaaggaggagactagcaggctgcttgccaaccctgagcatgtatcctaccagtgtgtgggcctcacaccagacaaactagtgaggcatagtgtgatgagagagaaacgaaggttacagagtggtaaaagagacagtgtgactcctggttagaggatagctgagagggccatcatgagaggtactcagaaggactaaagggcaaagtgagaggaggcctttaagacagagagtagatgggtagatgaatggacagggagagagatggttggttagcagataatagagaaatgatagacagatagacagacagacagatgatggatagacacatagaacaagacaaatgataaatgaatagatgatagacaaaggagatagagagacagaagcaagttgaatgggcaggaagataaagtcaggaagacacagagctctggtcaagaacccaggggagagcagaccagggagaagaggagagtgaactcctcgggggagtgtaactctagaaatcagaaaaaaacaaaaaaaaaaaaccccaaaaaacaaacaaacaaacaaacaaaaaaattggatacaggcaggaagaaggaagagatagagactgggagaaactagacacagaaccagtcaaagaagcagagggagagagacccatggcgggaataaagagaagcagaaacccagacacaaggcttcagcaaagctgggccagtgccagacatgccccgaacgaacgacagaggagtcacccagtactgttgcctgggaacagagtggagaaggaactaagaggcagccagccagctagacacataacaggaagagaaagaaggactcagggagaggctggctcctctcagtgggggtagttccaaattctggagctgcagtcacccaggccctctacctttcctgaacctagtagatccattcctaggcctgctcactcaccttgttcctcctcagctgagcaactcatggaacaacgttggtagaaaggagagagagtctgaggagcaccaggcttgaccttaactgacaccgggctctcatgggcctggcctcagtctcaggtgtcaatcacccccctcaaatgtctggcgcacatggagaaactgaggtccacagaggaagacagattccaggaaccttctcttcccagtcaccacccccactgctcccccagacccagactctttctcttccaaatcctgtttctgcatcacctggcacaggacaatggtggtaaccctcccgtgaggacttcctcctaatttcctccttccacacttaccgccacaaagaacatggtgaagaggtagaccatggcctccatgtagaaacgcctcttggtagcgatgctcactgtcgggaggaaggccaggctgctgagggtaggcaggagcagtttggctacaactgtccccatggaccaggaggaaggcactgactggggagaaggtggtaaaggcccccctggtctccagggcaggaagaaaaagagcccacttctttgcttctccagcagccctgaccgcagctgtggcagcacccacaaggagggcttaagtgctc

SEQ ID NO: 65 - DNA, 10526 bp, synthetic construct
  misc_feature 1..10526: note = Myomaker - Mouse (- strand, reverse complement)
  source 1..10526: mol_type = other DNA
gagcacttaagccctccttgtgggtgctgccacagctgcggtcagggctgctggagaagcaaagaagtgggctctttttcttcctgccctggagaccaggggggcctttaccaccttctccccagtcagtgccttcctcctggtccatggggacagttgtagccaaactgctcctgcctaccctcagcagcctggccttcctcccgacagtgagcatcgctaccaagaggcgtttctacatggaggccatggtctacctcttcaccatgttctttgtggcggtaagtgtggaaggaggaaattaggaggaagtcctcacgggagggttaccaccattgtcctgtgccaggtgatgcagaaacaggatttggaagagaaagagtctgggtctgggggagcagtgggggtggtgactgggaagagaaggttcctggaatctgtcttcctctgtggacctcagtttctccatgtgcgccagacatttgaggggggtgattgacacctgagactgaggccaggcccatgagagcccggtgtcagttaaggtcaagcctggtgctcctcagactctctctcctttctaccaacgttgttccatgagttgctcagctgaggaggaacaaggtgagtgagcaggcctaggaatggatctactaggttcaggaaaggtagagggcctgggtgactgcagctccagaatttggaactacccccactgagaggagccagcctctccctgagtccttctttctcttcctgttatgtgtctagctggctggctgcctcttagttccttctccactctgttcccaggcaacagtactgggtgactcctctgtcgttcgttcggggcatgtctggcactggcccagctttgctgaagccttgtgtctgggtttctgcttctctttattcccgccatgggtctctctccctctgcttctttgactggttctgtgtctagtttctcccagtctctatctcttccttcttcctgcctgtatccaatttttttgtttgtttgtttgtttgttttttggggttttttttttttgtttttttctgatttctagagttacactcccccgaggagttcactctcctcttctccctggtctgctctcccctgggttcttgaccagagctctgtgtcttcctgactttatcttcctgcccattcaacttgcttctgtctctctatctcctttgtctatcatctattcatttatcatttgtcttgttctatgtgtctatccatcatctgtctgtctgtctatctgtctatcatttctctattatctgctaaccaaccatctctctccctgtccattcatctacccatctactctctgtcttaaaggcctcctctcactttgccctttagtccttctgagtacctctcatgatggccctctcagctatcctctaaccaggagtcacactgtctcttttaccactctgtaaccttcgtttctctctcatcacactatgcctcactagtttgtctggtgtgaggcccacacactggtaggatacatgctcagggttggcaagcagcctgctagtctcctccttagagcagagccaaacttttagagactagcatcctctccttaggcctgcccttcctgcagcaggtctcagtaaggcaagggcatagagtatgtgaaggtatccagctggctctcaatgagtgagcccacaaactcacacatctgtgctcacatgcgtgttccatatcctgagtcagctggcatgactttctagtggtgggagaagccacaatgcatgtgggctgagaacagtgggggagggcttggcacctgtctacctcctggttgtggtggtcccataggtaacccaaggaactggaaactctatggctcttgagttcacttcagtaggggaggacattaggccaatgataagtcacaagaaagcaaccatggtggggttggactcattatcacccacgagcctaacatagtgatttcaatttgatagaagaggaaactgagtctcagagaaactgggccaccagtgtcaccatgaacactcagatcctggtctgccccacagtactttgtcccacactgtcatttgttcctcttgagacctggccaaggtcagagccaagatgagaccccacggtcaaggacataagccagggtcttgttcccaaggcctgtgttagatacagtccagcaaatcacagccccaatcaggtcacccctgcctgcctgggtctaattggcctacagctgcctctgcactggccttggaggcccaccctgccacaccccacccagagtggcagggccagctgtctcttatgacaaatgtcctctggcctcaaagccacaatctgttcctcacagagttctgccttccacgtggctgctgtaggactctccatgacaactaccagttgtatggtatgctgctgctgaatagaagaatgactcttggtgtcagttacacagcgggtggatctgatgtattccaaagaattctgccctctcctgttctaacctgatagtcatctaatctaaaatcaggttctaatctaagaatcttagacaatatcatcctttctacttgctgaacagcacaacaaacagggacaaaaagaatgggatctgagtcttaggcttttatagcagacagctgtctctctggccctttgactcagtagcacacaaatccacaatcagatattatcagcctacacccacattttgctttcaacatggtctccataccttgctgtttctaacacacgtggtcttagacctggtcaccacatctcacacaaacatatactgttctgagtcgggcatgaaagagtcacaaagactcactagagtcctccaccagaaatgcaaagcataataagatcgattgaattgtttttcccagaggtgagctaattctgcccagggcaagcacattgtttaaatgcccataacgcacatattaacttggtttcaggttgggggaaagtttgattaatgaaagcaaactttaaacagcatttcatttttgcagtgtggggtgccatgctccgcagttatcgttagggtccccttgtaagccccacagaacaggtgttctcatgccattagacaaggtgggcctgagagacctgagagaacctgggcccctctgccagctctgagctgacagcagggttagggctcctgtcacacccagctgtgtcctagcctggcaccagctggaccagatctccctgcctctggggagaaagggtacacatcacagccttgcccctgcctccttgggcaggaggttccccagggaagttcactgtcacacaggtcacccaccccccaaaaaattaatcctcagggcctgaggacagttagatcccttgttagaaagcctgctcctctggccttcacatgtagccaagtattctatgttgagatcaagcctaaggaagctcttctcctcgtgggggaaggcatgagtgtttcccaggatctcacagtaagtaagttttactcattcatgggggcctatacaagagaaggaagcaagatgctacagatgatgggctcaggtggggtggggtggggtcatgtggttctgtaaggagccagaagagcagagtcccctcccagagctgagttcctttccttctccacttgcgtaccttggtctggcccaacccaaagcttgtcttttcctgagctcatacctagttggttaacctcctcttcaccaatctcccttttaaaaggtgcagaacccaaagctcaaggctggggctgacccaacacagaggctggaccacctcctcccttcccctggatgctctctattgattgacagagtccatgtgcaactgtgaccagcaggaggtctctgagcttctaagtaggccctatgtgcttgactgatacatccatcatccagggtccccagctctccgcctgcctccctcggtggtgcccctgctgcctccagacaaggctgttttccagcttgcctgctccctcctgctaagttgggcttaccaagagctcattgtgctggctgctgggcttgtttgtgccagttgcacttgtcaaaataattatgtcatgtaattaaatattacttaaaatgatgaaatgtgaagcaaagggagagcaagttgttttctgcaagaaataagttgtctgcttggaaatcctgcatatagaaccttttgcttagaagcaaatctattcaactacgagtcagggacacacctgctggcatatgggggaaagaaaccagtgtgtcagaatcagcacttgcttggggggaatctaagggcttcctcttttatggagagacaggggtccaggataaaaggctcctatgcaaagactggcataggaatgtgtacactttcagtcagtcatgggcaaaggtgtaagtggtctttaaggatgcccttctgagcatgcttctcaccagccttgggccagtgctgagtctgaaagggatatttacaaagacttttgcactcccaggctagatggactcacctgtttaatctccacaagggctctgatagtgtgagggaggaggctgaggtacaaaaccattaggggctcacagctagtgaacctgagccttgggaccagttctcacccactcctgggctgcccactgcctgctgacctcatgtgatttccctacagttctcccatgcctgtgatgggcctggtttgtctgtgctgtgcttcatgcgccgtgacattctggagtacttcagcatctatggaacagccctgagcatgtgggtctccctgatgggtaagtggccatcttggccaatgggtgggagccagtcctgaaccccagccagtacccagcccctctctgagatcctccctccttgctgctttgcagagcttaatctgcttaaagagacatgcacatttctctgatgcctgcactctcatttccaccatccttaagtgactccagtagttagcacttgtgacatttaaaaaacagaagcatacaaaggagaggccaaaggcatcctggacctagcctcccagcttgtcctccaggctcagaggagcatttgccctcatgggtcagctcagctctgtgtattaggaaggcagaccattcaaaatcctcaccttggacctggggtatatacagctcaatggcagatcgctcgcctggtaatcaataggcccttcattccattaccagcaactgcaaaattttgaaagaaaaagaaggaagagatagagaaaagtagaaagcagaaaggatgaaggaagaagaaaggaaaggagacagggagggagggaggaagggagacagggagagaaggagggagagagcaaagaaaggggaaagaaagggaagggaaggaaagagaaaagggagaaaccaagcaagctcacccttgtctcccagggatgcagtcccggggtccctcctgagactcagctctgcgcaccaatcattagtcttaacacttttgtctcaggattcctaggaaatgctggtcactcagtctaccagtttatttcagccaccctgctccagggaagcagcatcacccactccctccaaataaccaaaattcagaccttatggaaaccaggctggccctacagattgagaggacataccaataggttcccaaggatggaggcacagccatgtgagggacgctgctcaccatagctatgcctctccccagcactggccgactttgatgaaccccagagatcgaccttcacaatgcttggcgtccttaccatcgctgtgcggacttttcatgaccgctggggttacggggtatactccggtcccataggcacggccaccctcatcattgctgtaaagtgggtgagtacttccagtatctccactgtcggagaccacggaacctgcatttcttccctgatcttggtttctcctatgtagggtcctataccccatatccttatatgcaggtgaattagtaagaattgggccaaaaaccctaaaattcctaaaaatggtggctcatgctcgggtcccatgccctgctggtttattggtcctggataaagccaaaactccttttctcttgacctctgctctgcatccaaatacccataaagaatgcttctaagcacaggcacaggcacaggtgtgatttttaatatacccagagctgaggagaccttttgtcatcatgactgtcactgtcagtcttttcatcaacataagatcactatcattatcattctgagagacaacactgcttacaggtataataccagtttggagagcagataggttaatctggatagtcttcccgaaagaagcaagccttggaaatggttctcatgaggaaggaaggtgtgaggtgggggtgaagcagggtattgagtgggaggcctagaggagggcctggcgcttggcatctactctgctgtataggctcctaacccctctatggtctcaaggccctctcacctccatggcctaaaacccacctaagttagccatcgtgaacaaatttcccaatagcaggaaagacccagggatgttttctgagctccacccagagcagttaggcccaaaacacagaccttccaggccagcaggcttcagaccaagcagacagcactcaggcttcaagttctcacctgtctgctacctcatgcaggaagcaccatttgggatcttgcaggttcctggaagtagagctacagcagtgcagattggggcaggcggtggggtgtgtgtgtgtgtgtgtgcctttgtgtgtgtgtgtgcctttgtgtgtgtgtctgtgtgtgtctgtgtgtgtctgtgtgactgtgtgtctgagtctgagtctgagtctgagtctgagtctgagtctgagtctgagtctgagtctgtgtctgtgtctgtgtctgtgtctgtgtctgtgtctgagtctgtgtctgtgtctgtgtctgtgtctgtgtctgtgttgtctgtgtctgtgtctctgtgtctgtgtctatgtctgtgtctgtgtctgtgtctgtgtctgtctgtgtctgtgtcgtctgtgtctgtgtctgtgtctgtgtctgtgtctgtgtctgtctgtgtctgtgtctgtctgtgtctgtgtctgtgtctgtctgtgtctgtgtcgtctgtgtctgtgtctgtgtctgtgtcgtctgtgtctgtgtctgtctgtgtctgtgtctgtctgtgtctgtgtcgtctgtgtctgtgtctgtgactgtgtctgtgtcgtctgtgtctgtgtcatctgtgtctgtgtctgtgtctgtgtctgtgtctgtgtctgtgtctgtgtctgtgtctgtgtctgtctgtgtctgtgtcgtctgtgtctgtgtctgtgtctgtgtctgtctgtgtctgtgtcgtctgtgtctgtgtctgtgtctgtgtctgtctgtgtctgtgtctgtctgtgtctgtgtctgtctgtgtctgtgtcgtctgtgtctgtgtctgtgtctgtgtctgtgtctgtgtctgtgtctgtgtctgtgtctgtgtctgtgtctgtgtctgtgtctgtctgtgtctgtgtctatgcctgtgtgtctgtgtctgtgtctgtgtctgtgtctgtgtctgtgtctgtgtctgtgtctgtgtctgtgtctgtgtctgtgtctgtctgtgtctgtgtctgtctgtgtctgtgtctgtgtctgtgtctgtgtctgtgtctgtgtctgtgtctgtgtctgtgtctgtgtctgtgtctgtgtctgtgtcagaggggagtggcagggccaggggtgggagagctctgatccatcttcagcaaagtggggacaggtatagtcagggaggaagcttccaagccacatcctactcctgtgggctccgaggaacccgggcttattctgattttaagttaaggatgaacctgaaatgcacagagctcagcagcctaacctgcagccctagtaggtaatggcagctgtgcttgactttcgaggggagaagcttccatcccactccagtttgaggagccgaagctggccctctctgacccaaggcagaggtgttgggcttctgcatggctagttaacaagctggaatgcataaacaagaaggcttgctctgataactgcctctttgtcttgcctatcatggccccttgctgctcttcactggttctggatctgacttgattgtttgtttgtttgtttgtttgtttgtttgtttttaaagatagactctcactttgtatctctggatggcttcaaactcatagagatctgcccgcctctgcctcttgaatgctggtgtccaagcccagcacacccatcctgatgggattttaattagccaggatagcatacatgtgccagtgcccccctccactaaatgccagcctccccaggtctctggtgagaatgggagtgaggggctgcagccacccatgcctggggcacagaccccatctcctagatcttagataggcaggtggtttggacttacttcttagaacggagtacaattctttcccatgtctcaccctttcaggaaaggaacatgaatacaacatttggggagaagaagctgagtgaaatgggaaataggggttcccggggcaagacagggcccatgggtgatcttcaatattcttctcctctctggggccccagtgttagaactgtgtgattgatggtcatacggcctacactcaggctaataggcggtgcccatgtcactggcactgctcactgggacctccactcctgttactaatggcaagttttagaacacttggaaacagcaacatatcatcactcagagtgacaaagcttgccctgatttgcacgaggccattgacagcatttgtacatataatgtatttagtgaggtgtgcaattagggccgctgtcctgtgcccactgtgcacatcactcagtcagggctgctgtcctgtgccctctgtgcacacctgacagtggtatttataatgatcttccccactgaaacctgaacaatcttgaatacctaaaatacctttgggccccaaggatgtgcattccagtgaggaaccatgggactcccatctattccatgtaacactccatcttaccaagcttgaacacacagggcctatgaaaccaaggttaacagaggaaaaccccttagctgggaaaactgatcacgtctgccactgaagtgccaaagcccaccagatgcgggcagtagaggacccaggggaaattggcccagagagtcccatcagtcaggcatacagaggaatgggggtagggctcttctacagttcatggaggggtcccttcctgtgctgcaccccaagaactttgatgtccccaccttgtgcctgcagctgaagaagatgaaagagaagaagggcctgtaccccgacaagagcatctacacccagcagataggccccggcctgtgctttggggccctggccctgatgcttcgattcttctttgaggtacctggcctatggggaaggggagcaagagcctctggaaatagttaactaacagccacatatggaggctccaagttgtaaattctgtcctcttgaggatggtactcaccatccccagtgtactagcctcactgcctgagtggacaagtcaggccctgactttaggaagcctgcacccaagatgcacgcatgtcctggaaggaaccaggagctggtgcccagcacccaggaggcatggaacagaggaaggcagcaagcctttctgccaccttctcagggtgggctggctgacagaggcaccaaatggctaggacttggtttagggaagggatggaggcccagactgactcattctcctccacaggaatgggattacacctacgtccacagcttctaccactgtgccctggccatgtcctttgtcctgctgctgcccaaggtcaacaagaaggctgggaacgcaggggcccccgccaagctgaccttctccaccctctgctgcacttgtgtctgactatacccccccacacacacacacacaccaggcccctgccttcctgcctggcagtcctgctgtctctcccaaggtacttcctatactttgttatgcggcctgtacatgagaaatggtcttctctacaccccaagagaccagcaggcctgctgcattctgctgagtgctgcttagggacccactggttctgtgttcaccagttgcttcactctgttcaggaaaaaaaagaactttatcccccaaggcctcacaaccataggtgtgcctggcagagaaccctagaccagtaaatacccagcagcatgcagggttatctatttcccaggtcctgcctgtcagaatcgtctgctttccctaggaaactgggattgcccttttaacccctgcccaggctctgaaagctctccacttaggaagctggagccagcgaaccttgcatacccctgcctgagtcccatcccttctgcaggttttcgatcaagccattcacagtaaactcttgatcagccactagtcattagcttcgcctaacatacattctagttcctggaa